European Patent Specification EP 3 988 112 B1, published August 13, 2025. Title: Compounds, Compositions, Methods, and Kits Relating to Telomere Extension. Applicant: THE BOARD OF TRUSTEES OF THE LELAND STANFORD JUNIOR UNIVERSITY. The sequence listing filed with the application follows.

SEQUENCE LISTING (10 sequences)

SEQ ID NO: 1 - DNA, 20 bp, Artificial Sequence
  PCR Primer
gccctcagacttcaagacca

SEQ ID NO: 2 - DNA, 20 bp, Artificial Sequence
  PCR Primer
aggcagaatccagatgctca

SEQ ID NO: 3 - DNA, 20 bp, Artificial Sequence
  PCR Primer
gtggacctgacctgccgtct

SEQ ID NO: 4 - DNA, 20 bp, Artificial Sequence
  PCR Primer
ggaggagtgggtgtcgctgt

SEQ ID NO: 5 - DNA, 20 bp, Artificial Sequence
  PCR Primer
gtcacctacgtgccactcct

SEQ ID NO: 6 - DNA, 19 bp, Artificial Sequence
  PCR Primer
agcaagaaagcgagccaat

SEQ ID NO: 7 - DNA, 20 bp, Artificial Sequence
  PCR Primer
gccctcagacttcaagacca

SEQ ID NO: 8 - DNA, 19 bp, Artificial Sequence
  PCR Primer
gctgctggtgtctgctctc

SEQ ID NO: 9 - DNA, 20 bp, Artificial Sequence
  PCR Primer
caatgaccccttcattgacc

SEQ ID NO: 10 - DNA, 20 bp, Artificial
  PCR Primer
ttgattttggagggatctcg